European Patent Specification EP 3 727 451 B1, published May 10, 2023. Title: RECOMBINANT PSEUDOMONAS AERUGINOSA LYSINS. Applicant: THE ROCKEFELLER UNIVERSITY. The sequence listing filed with the application follows.

SEQUENCE LISTING (29 sequences)

SEQ ID NO: 1 - protein, 143 aa, Pseudomonas aeruginosa phage
MRTSQRGIDLIKSFEGLRLSAYQDSVGVWTIGYGTTRGVTRYMTITVEQAERMLSNDLQRFEPELDRLVKVPLNQNQWDALMSFVYNLGAANLESSTLRRLLNAGDYAGAAEQFLRWNKAGGKVLPGLVRRRASERELFLGAA

SEQ ID NO: 2 - protein, 144 aa, Pseudomonas aeruginosa phage
MRTSQRGIDLIKSFEGLRLSAYQDSVGVWTIGYGTTRGVTRYMTITVEQAERMLSNDLQRFEPELDRLVKVPLNQNQWDALMSFVYNLGAANLASSTLLKLLNKGDYQGAADQFPRWVNAGGKRLEGLVKRRAAERALFLESLS

SEQ ID NO: 3 - protein, 144 aa, Pseudomonas aeruginosa phage
MRTSQRGIDLIKGFEGLRLSAYQDSVGVWTIGYGTTRGVTRYMTITVEQAERMLSNDLRRFEPELDRLVKAPLNQNQWDALMSFVYNLGAANLASSTLLKLLNKGDYQGAADQFPRWVNAGGKRLEGLVKRRAAERVLFLEPLS

SEQ ID NO: 4 - protein, 144 aa, Pseudomonas aeruginosa phage
MRTSQRGIDLIKSFEGLRLSAYQDSVGVWTIGYGTTRGVTRYMTITVEQAERMLSNDIQRFEPEMDKLVKVPLNQNQWDALMSFVYNLGAANLASSTLLKLLNKGDYQGAADQFPRWVNAGGKRLEGLVKRRAAERVLFLEPLS

SEQ ID NO: 5 - protein, 144 aa, Pseudomonas aeruginosa phage
MRTSQRGIDLIKSFEGLRLSAYQDSVGVWTIGYGTTRGVTRYMTITVEQAERMLSNDLQRFEPELDRLVKVPLNQNQWDALMSFVYNLGAANLASSTLLKLLNRGDYQGAADQFSRWVNAGGKRLGGLVKRRAAERVLFLEPLS

SEQ ID NO: 6 - protein, 144 aa, Pseudomonas aeruginosa phage
MRTSQRGIDLIKSFEGLRLSAYQDSVGVWTIGYGTTRGVTRYMTITVEQAERMLSNDLQRFEPELDRLVKVALNQNQWDALMSFVYNLGAANLASSTLLKLLNKGDYQGAAEQFPRWVNAGRKRLEGLVKRRAAERALFLEPLS

SEQ ID NO: 7 - protein, 144 aa, Pseudomonas aeruginosa phage
MNISKAGLDLIKEFEGLRLSAYQDSVGVWTIGYGHTRTAKRGMSITSDQADALLIADLADAEDDVERYVRQDMRQNEFDALVSLVFNIGGSNFSRSTMLRLINEKAEAWKIGAEFLKWVYAKGRKLPGLERRRLAERNLYLKGA

SEQ ID NO: 8 - protein, 153 aa, Pseudomonas aeruginosa phage
MKLPRKLTAAGGALALAAALVTPFEGRSLVAYRDPVGIPTICEGITAGVRMGDMATPAECDALLKRELQRAVDAVDRQVLVPLPDTRRAALASFVYNVGEGQLARSTLLRKLNAGDVRGACAELSRWVYAGGKKLGGLVRRRAAERELCEVGL

SEQ ID NO: 9 - protein, 153 aa, Pseudomonas aeruginosa phage
MKLPPKLAAGGGVLALAAALVAPFEGRSLVAYLDPVGIPTICEGITAGVRMGDRATQAECDALLERELQRAVDAVDRQVLVPLPDTRRAALGSFVYNVGEGQLARSTLLRKLNAGDVRGACAELSRWVYAGGKKLGGLVRRRAAERELCEIGL

SEQ ID NO: 10 - protein, 150 aa, Pseudomonas aeruginosa page
MKTWQRVTGALAIASALVAAHEGRSLVAYIDPVGIPTICEGITAGVRLGDRATPQQCDALLETEVRKSLSSVERLATVQMPDTRKAALASFVYNVGETQFSRSTLLRKLNAGDVKGACAELSRWVYAGGKVYKGLVNRRKAERELCERGL

SEQ ID NO: 11 - protein, 166 aa, Pseudomonas aeruginosa phage
MIRPPQRRTVAALTLSAAALVGIVLHEGYTDRAVIPVKGDVPTIGFGTTTGVKLGDTTTPPKALARALTDVQQFEGALKQCVTVPLAQHEYDALVSFSYNVGSRAFCQSTLVRKLNAEDYAGACAELLRWRFFQGKDCAQPANARLCGGLVTRREAEYRQCIGETP

SEQ ID NO: 12 - protein, 145 aa, Pseudomonas aeruginosa phage
MAKRFEGFHRVPKSDPLRRAHPYICPAGYWTIGYGRLCKPDHPPISEDEGEAYLRQDLRTALAATLRYCPVLATEPEGRLAAIADFTFNLGAGRLQTSTLRRRINQRDWPAAATELRRWVYGGGKVLPGLVTRREAEVALLLRNA

SEQ ID NO: 13 - protein, 154 aa, Pseudomonas aeruginosa phage
MKGKVIGGSAAAVIALAAAALVKPWEGYSPTPYIDMVGVATHCYGDTSRADKAVYTEQECAEKLNSRLGSYLTGISQCIKVPLREREWAAVLSWTYNVGVGAACRSTLVGRINAGQPAASWCPELDRWVYAGGKRVQGLVNRRAAERRMCEGRS

SEQ ID NO: 14 - protein, 172 aa, Pseudomonas aeruginosa phage
MLAVLAGTGFTLTSQDLPAPIERAAITAGLMVLTPEMEGTRFKAYPDTGGVWTICTGRTQGVKRGDQATPDECAAYLRADLGASVDFVLRERPKVSLLCKVAIADMHYNTGPGAVGRSTLLVKAKAGDQVGAAEQFRRWVYVGGQDCRLASSNCGGIINRREIQRSLCLVNQ

SEQ ID NO: 15 - protein, 170 aa, Pseudomonas aeruginosa phage
MASRKYLSAAVLALIAASASAPAIMDQFIREKEGESLKAYQDGARVWTICNGKTAGVTRSTTMTKAECDAWRRTEIGQRLEFVHSIITVRMSEPAWAGVGSWCFNVGNKACAGSTAVRLLNAGNQPAGCRAMLSWRFITRDGKKVDCSTPQPYCSGVWERRQGEAELCSL

SEQ ID NO: 16 - protein, 174 aa, Pseudomonas aeruginosa phage
MKLAWGKKVDQAFRDKVFAICDGFKWNRETHASWLMSCMAFESGETFSPSVRNAAGSGATGLIQFMPRTAQGLGTSTAELAAMSAVDQLDYVQKYFRPYASRIGTLSDMYMAILMPKFVGQPEDSVLFLDPKISYRQNAGLDANRDGKITKAEAASKVRAKFDKGMLDRFALEL

SEQ ID NO: 17 - protein, 220 aa, Pseudomonas aeruginosa phage
MKITKDVLITGTGCTTDRAIKWLDDVQAAMDKFHIESPRAIAAYLANIGVESGGLVSLVENLNYSAQGLANTWPRRYAVDPRVRPYVPNALANRLARNPVAIANNVYADRMGNGCEQDGDGWKYRGRGLIQLTGKSNYSLFAEDSGMDVLEKPELLETPAGASMSSAWFFWRNRCIPMAESNNFSMVVKTINGAAPNDANHGQLRINRYLKTIAAINQGS

SEQ ID NO: 18 - protein, 174 aa, Pseudomonas aeruginosa phage
MAWSAKVSQAFCDRVIWIAASLGMPADGADWLMACIAWETGETFSPSVRNGAGSGATGLIQFMPATARGLGTTTDELARMTPEQQLDYVYRYFLPYRGRLKSLADTYMAILWPAGIGRALDWALWDSTSRPTTYRQNAGLDINRDGVITKAEAAAKVQAKLDRGLQPQFRRAAA

SEQ ID NO: 19 - protein, 224 aa, Pseudomonas aeruginosa phage
MKLAWGKKVDQAFRDKVFAICDGFKWNRETHASWLMSCMAFESGETFSPSVRNAAGSGATGLIQFMPRTAQGLGTSTAELAAMSAVDQLDYVQKYFRPYASRIGTLSDMYMAILMPKFVGQPEDSVLFLDPKISYRQNAGLDANRDGKITKAEAASKVRAKFDKGMLDRFALELGTGGGSGGGSGGGLLGDFFRKSKEKIGKEFKRIVQRIKDFLRNLVPRTES

SEQ ID NO: 20 - protein, 214 aa, Pseudomonas aeruginosa phage
MKLAWGKKVDQAFRDKVFAICDGFKWNRETHASWLMSCMAFESGETFSPSVRNAAGSGATGLIQFMPRTAQGLGTSTAELAAMSAVDQLDYVQKYFRPYASRIGTLSDMYMAILMPKFVGQPEDSVLFLDPKISYRQNAGLDANRDGKITKAEAASKVRAKFDKGMLDRFALELGTGGGSGGGSGGGDHECHYRIKPTFRRLKWKYKGKFWCPS

SEQ ID NO: 21 - protein, 205 aa, Pseudomonas aeruginosa phage
MKLAWGKKVDQAFRDKVFAICDGFKWNRETHASWLMSCMAFESGETFSPSVRNAAGSGATGLIQFMPRTAQGLGTSTAELAAMSAVDQLDYVQKYFRPYASRIGTLSDMYMAILMPKFVGQPEDSVLFLDPKISYRQNAGLDANRDGKITKAEAASKVRAKFDKGMLDRFALELGTGGGSGGGSGGGRKKTRKRLKKIGKVLKWI

SEQ ID NO: 22 - protein, 211 aa, Pseudomonas aeruginosa phage
MKLAWGKKVDQAFRDKVFAICDGFKWNRETHASWLMSCMAFESGETFSPSVRNAAGSGATGLIQFMPRTAQGLGTSTAELAAMSAVDQLDYVQKYFRPYASRIGTLSDMYMAILMPKFVGQPEDSVLFLDPKISYRQNAGLDANRDGKITKAEAASKVRAKFDKGMLDRFALELGTGGGSGGGSGGGRRWVRRVRRWVRRVVRVVRRWVRR

SEQ ID NO: 23 - protein, 205 aa, Pseudomonas aeruginosa phage
MKLAWGKKVDQAFRDKVFAICDGFKWNRETHASWLMSCMAFESGETFSPSVRNAAGSGATGLIQFMPRTAQGLGTSTAELAAMSAVDQLDYVQKYFRPYASRIGTLSDMYMAILMPKFVGQPEDSVLFLDPKISYRQNAGLDANRDGKITKAEAASKVRAKFDKGMLDRFALELGTGGGSGGGSGGGALYKKFKKKLLKSLKRKG

SEQ ID NO: 24 - protein, 209 aa, Pseudomonas aeruginosa phage
MKLAWGKKVDQAFRDKVFAICDGFKWNRETHASWLMSCMAFESGETFSPSVRNAAGSGATGLIQFMPRTAQGLGTSTAELAAMSAVDQLDYVQKYFRPYASRIGTLSDMYMAILMPKFVGQPEDSVLFLDPKISYRQNAGLDANRDGKITKAEAASKVRAKFDKGMLDRFALELGTGGGSGGGSGGGGIGKFLKKAKKFGKAFVKILKK

SEQ ID NO: 25 - DNA, 39 bp, artificial sequence
  PCR primer
aattcgtcgacggggcggccgcggtacctctagactgca

SEQ ID NO: 26 - DNA, 31 bp, artificial sequence
  PCR primer
gtctagaggtaccgcggccgccccgtcgacg

SEQ ID NO: 27 - protein, 4 aa, artificial sequence
  Cloning sequence
GPVD

SEQ ID NO: 28 - protein, 12 aa, artificial sequence
  Linker sequence
GGGSGGGSGGGG

SEQ ID NO: 29 - protein, 144 aa, Pseudomonas aeruginosa phage
MRTSQRGIDLIKSFEGLRLSAYQDSVGVWTIGYGTTRGVTRYMTITVEQAERMLANDIQRFEPELDKLVKVPLNQNQWDALMSFVYNLGSANLASSTLLKLLNKGDYRGAADQFPRWVNAGGKRLEGLVKRRAAERALFLEPLS